European Patent Application EP 4 180 526 A2, published May 17, 2023. Title: Composition for cleaving a target DNA comprising a guide RNA specific for the target DNA and Cas protein-encoding nucleic acid or Cas protein, and use thereof. Applicant: TOOLGEN INCORPORATED. The sequence listing filed with the application follows.

SEQUENCE LISTING (111 sequences)

SEQ ID NO: 1 - DNA, 4107 bp, Artificial Sequence
  Cas9-coding sequence
atggacaagaagtacagcatcggcctggacatcggtaccaacagcgtgggctgggccgtgatcaccgacgagtacaaggtgcccagcaagaagttcaaggtgctgggcaacaccgaccgccacagcatcaagaagaacctgatcggcgccctgctgttcgacagcggcgagaccgccgaggccacccgcctgaagcgcaccgcccgccgccgctacacccgccgcaagaaccgcatctgctacctgcaggagatcttcagcaacgagatggccaaggtggacgacagcttcttccaccgcctggaggagagcttcctggtggaggaggacaagaagcacgagcgccaccccatcttcggcaacatcgtggacgaggtggcctaccacgagaagtaccccaccatctaccacctgcgcaagaagctggtggacagcaccgacaaggccgacctgcgcctgatctacctggccctggcccacatgatcaagttccgcggccacttcctgatcgagggcgacctgaaccccgacaacagcgacgtggacaagctgttcatccagctggtgcagacctacaaccagctgttcgaggagaaccccatcaacgccagcggcgtggacgccaaggccatcctgagcgcccgcctgagcaagagccgccgcctggagaacctgatcgcccagctgcccggcgagaagaagaacggcctgttcggcaacctgatcgccctgagcctgggcctgacccccaacttcaagagcaacttcgacctggccgaggacgccaagctgcagctgagcaaggacacctacgacgacgacctggacaacctgctggcccagatcggcgaccagtacgccgacctgttcctggccgccaagaacctgagcgacgccatcctgctgagcgacatcctgcgcgtgaacaccgagatcaccaaggcccccctgagcgccagcatgatcaagcgctacgacgagcaccaccaggacctgaccctgctgaaggccctggtgcgccagcagctgcccgagaagtacaaggagatcttcttcgaccagagcaagaacggctacgccggctacatcgacggcggcgccagccaggaggagttctacaagttcatcaagcccatcctggagaagatggacggcaccgaggagctgctggtgaagctgaaccgcgaggacctgctgcgcaagcagcgcaccttcgacaacggcagcatcccccaccagatccacctgggcgagctgcacgccatcctgcgccgccaggaggacttctaccccttcctgaaggacaaccgcgagaagatcgagaagatcctgaccttccgcatcccctactacgtgggccccctggcccgcggcaacagccgcttcgcctggatgacccgcaagagcgaggagaccatcaccccctggaacttcgaggaggtggtggacaagggcgccagcgcccagagcttcatcgagcgcatgaccaacttcgacaagaacctgcccaacgagaaggtgctgcccaagcacagcctgctgtacgagtacttcaccgtgtacaacgagctgaccaaggtgaagtacgtgaccgagggcatgcgcaagcccgccttcctgagcggcgagcagaagaaggccatcgtggacctgctgttcaagaccaaccgcaaggtgaccgtgaagcagctgaaggaggactacttcaagaagatcgagtgcttcgacagcgtggagatcagcggcgtggaggaccgcttcaacgccagcctgggcacctaccacgacctgctgaagatcatcaaggacaaggacttcctggacaacgaggagaacgaggacatcctggaggacatcgtgctgaccctgaccctgttcgaggaccgcgagatgatcgaggagcgcctgaagacctacgcccacctgttcgacgacaaggtgatgaagcagctgaagcgccgccgctacaccggctggggccgcctgagccgcaagcttatcaacggcatccgcgacaagcagagcggcaagaccatcctggacttcctgaagagcgacggcttcgccaaccgcaacttcatgcagctgatccacgacgacagcctgaccttcaaggaggacatccagaaggcccaggtgagcggccagggcgacagcctgcacgagcacatcgccaacctggccggcagccccgccatcaagaagggcatcctgcagaccgtgaaggtggtggacgagctggtgaaggtgatgggccgccacaagcccgagaacatcgtgatcgagatggcccgcgagaaccagaccacccagaagggccagaagaacagccgcgagcgcatgaagcgcatcgaggagggcatcaaggagctgggcagccagatcctgaaggagcaccccgtggagaacacccagctgcagaacgagaagctgtacctgtactacctgcagaacggccgcgacatgtacgtggaccaggagctggacatcaaccgcctgagcgactacgacgtggaccacatcgtgccccagagcttcctgaaggacgacagcatcgacaacaaggtgctgacccgcagcgacaagaaccgcggcaagagcgacaacgtgcccagcgaggaggtggtgaagaagatgaagaactactggcgccagctgctgaacgccaagctgatcacccagcgcaagttcgacaacctgaccaaggccgagcgcggcggcctgagcgagctggacaaggccggcttcatcaagcgccagctggtggagacccgccagatcaccaagcacgtggcccagatcctggacagccgcatgaacaccaagtacgacgagaacgacaagctgatccgcgaggtgaaggtgatcaccctgaagagcaagctggtgagcgacttccgcaaggacttccagttctacaaggtgcgcgagatcaacaactaccaccacgcccacgacgcctacctgaacgccgtggtgggcaccgccctgatcaagaagtaccccaagctggagagcgagttcgtgtacggcgactacaaggtgtacgacgtgcgcaagatgatcgccaagagcgagcaggagatcggcaaggccaccgccaagtacttcttctacagcaacatcatgaacttcttcaagaccgagatcaccctggccaacggcgagatccgcaagcgccccctgatcgagaccaacggcgagaccggcgagatcgtgtgggacaagggccgcgacttcgccaccgtgcgcaaggtgctgagcatgccccaggtgaacatcgtgaagaagaccgaggtgcagaccggcggcttcagcaaggagagcatcctgcccaagcgcaacagcgacaagctgatcgcccgcaagaaggactgggaccccaagaagtacggcggcttcgacagccccaccgtggcctacagcgtgctggtggtggccaaggtggagaagggcaagagcaagaagctgaagagcgtgaaggagctgctgggcatcaccatcatggagcgcagcagcttcgagaagaaccccatcgacttcctggaggccaagggctacaaggaggtgaagaaggacctgatcatcaagctgcccaagtacagcctgttcgagctggagaacggccgcaagcgcatgctggccagcgccggcgagctgcagaagggcaacgagctggccctgcccagcaagtacgtgaacttcctgtacctggccagccactacgagaagctgaagggcagccccgaggacaacgagcagaagcagctgttcgtggagcagcacaagcactacctggacgagatcatcgagcagatcagcgagttcagcaagcgcgtgatcctggccgacgccaacctggacaaggtgctgagcgcctacaacaagcaccgcgacaagcccatccgcgagcaggccgagaacatcatccacctgttcaccctgaccaacctgggcgcccccgccgccttcaagtacttcgacaccaccatcgaccgcaagcgctacaccagcaccaaggaggtgctggacgccaccctgatccaccagagcatcaccggtctgtacgagacccgcatcgacctgagccagctgggcggcgactaa

SEQ ID NO: 2 - protein, 21 aa, Artificial Sequence
  peptide tag
GGSGPPKKKRKVYPYDVPDYA

SEQ ID NO: 3 - DNA, 34 bp, Artificial Sequence
  F primer for CCR5
aattcatgacatcaattattatacatcggaggag

SEQ ID NO: 4 - DNA, 34 bp, Artificial Sequence
  R primer for CCR5
gatcctcctccgatgtataataattgatgtcatg

SEQ ID NO: 5 - DNA, 20 bp, Artificial Sequence
  F1 primer for CCR5
ctccatggtgctatagagca

SEQ ID NO: 6 - DNA, 21 bp, Artificial Sequence
  F2 primer for CCR5
gagccaagctctccatctagt

SEQ ID NO: 7 - DNA, 20 bp, Artificial Sequence
  R primer for CCR5
gccctgtcaagagttgacac

SEQ ID NO: 8 - DNA, 20 bp, Artificial Sequence
  F1 primer for C4BPB
tatttggctggttgaaaggg

SEQ ID NO: 9 - DNA, 24 bp, Artificial Sequence
  R1 primer for C4BPB
aaagtcatgaaataaacacaccca

SEQ ID NO: 10 - DNA, 24 bp, Artificial Sequence
  F2 primer for C4BPB
ctgcattgatatggtagtaccatg

SEQ ID NO: 11 - DNA, 21 bp, Artificial Sequence
  R2 primer for C4BPB
gctgttcattgcaatggaatg

SEQ ID NO: 12 - DNA, 20 bp, Artificial Sequence
  F1 primer for ADCY5
gctcccaccttagtgctctg

SEQ ID NO: 13 - DNA, 20 bp, Artificial Sequence
  R1 primer for ADCY5
ggtggcaggaacctgtatgt

SEQ ID NO: 14 - DNA, 21 bp, Artificial Sequence
  F2 primer for ADCY5
gtcattggccagagatgtgga

SEQ ID NO: 15 - DNA, 20 bp, Artificial Sequence
  R2 primer for ADCY5
gtcccatgacaggcgtgtat

SEQ ID NO: 16 - DNA, 20 bp, Artificial Sequence
  F primer for KCNJ6
gcctggccaagtttcagtta

SEQ ID NO: 17 - DNA, 20 bp, Artificial Sequence
  R1 primer for KCNJ6
tggagccattggtttgcatc

SEQ ID NO: 18 - DNA, 22 bp, Artificial Sequence
  R2 primer for KCNJ6
ccagaactaagccgtttctgac

SEQ ID NO: 19 - DNA, 20 bp, Artificial Sequence
  F1 primer for CNTNAP2
atcaccgacaaccagtttcc

SEQ ID NO: 20 - DNA, 20 bp, Artificial Sequence
  F2 primer for CNTNAP2
tgcagtgcagactctttcca

SEQ ID NO: 21 - DNA, 20 bp, Artificial Sequence
  R primer for CNTNAP2
aaggacacagggcaactgaa

SEQ ID NO: 22 - DNA, 20 bp, Artificial Sequence
  F1 primer for N/A Chr. 5
tgtggaacgagtggtgacag

SEQ ID NO: 23 - DNA, 22 bp, Artificial Sequence
  R1 primer for N/A Chr. 5
gctggattaggaggcaggattc

SEQ ID NO: 24 - DNA, 22 bp, Artificial Sequence
  F2 primer for N/A Chr. 5
gtgctgagaacgcttcatagag

SEQ ID NO: 25 - DNA, 23 bp, Artificial Sequence
  R2 primer for N/A Chr. 5
ggaccaaaccacattcttctcac

SEQ ID NO: 26 - DNA, 20 bp, Artificial Sequence
  F primer for deletion
ccacatctcgttctcggttt

SEQ ID NO: 27 - DNA, 20 bp, Artificial Sequence
  R primer for deletion
tcacaagcccacagatattt

SEQ ID NO: 28 - RNA, 105 nt, Artificial Sequence
  sgRNA for CCR5
ggugacaucaauuauuauacauguuuuagagcuagaaauagcaaguuaaaauaaggcuaguccguuaucaacuugaaaaaguggcaccgagucggugcuuuuuuu

SEQ ID NO: 29 - RNA, 44 nt, Artificial Sequence
  crRNA for CCR5
ggugacaucaauuauuauacauguuuuagagcuaugcuguuuug

SEQ ID NO: 30 - RNA, 86 nt, Artificial Sequence
  tracrRNA for CCR5
ggaaccauucaaaacagcauagcaaguuaaaauaaggcuaguccguuaucaacuugaaaaaguggcaccgagucggugcuuuuuuu

SEQ ID NO: 31 - DNA, 86 bp, Artificial Sequence
  Foxn1 #1 sgRNA
gaaattaatacgactcactataggcagtctgacgtcacacttccgttttagagctagaaatagcaagttaaaataaggctagtccg

SEQ ID NO: 32 - DNA, 86 bp, Artificial Sequence
  Foxn1 #2 sgRNA
gaaattaatacgactcactataggacttccaggctccacccgacgttttagagctagaaatagcaagttaaaataaggctagtccg

SEQ ID NO: 33 - DNA, 86 bp, Artificial Sequence
  Foxn1 #3 sgRNA
gaaattaatacgactcactataggccaggctccacccgactggagttttagagctagaaatagcaagttaaaataaggctagtccg

SEQ ID NO: 34 - DNA, 86 bp, Artificial Sequence
  Foxn1 #4 sgRNA
gaaattaatacgactcactataggactggagggcgaaccccaaggttttagagctagaaatagcaagttaaaataaggctagtccg

SEQ ID NO: 35 - DNA, 86 bp, Artificial Sequence
  Foxn1 #5 sgRNA
gaaattaatacgactcactataggaccccaaggggacctcatgcgttttagagctagaaatagcaagttaaaataaggctagtccg

SEQ ID NO: 36 - DNA, 86 bp, Artificial Sequence
  Prkdc #1 sgRNA
gaaattaatacgactcactataggttagttttttccagagacttgttttagagctagaaatagcaagttaaaataaggctagtccg

SEQ ID NO: 37 - DNA, 86 bp, Artificial Sequence
  Prkdc #2 sgRNA
gaaattaatacgactcactataggttggtttgcttgtgtttatcgttttagagctagaaatagcaagttaaaataaggctagtccg

SEQ ID NO: 38 - DNA, 86 bp, Artificial Sequence
  Prkdc #3 sgRNA
gaaattaatacgactcactataggcacaagcaaaccaaagtctcgttttagagctagaaatagcaagttaaaataaggctagtccg

SEQ ID NO: 39 - DNA, 86 bp, Artificial Sequence
  Prkdc #4 sgRNA
gaaattaatacgactcactataggcctcaatgctaagcgacttcgttttagagctagaaatagcaagttaaaataaggctagtccg

SEQ ID NO: 40 - DNA, 29 bp, Artificial Sequence
  F1 primer for Foxn1
gtctgtctatcatctcttcccttctctcc

SEQ ID NO: 41 - DNA, 25 bp, Artificial Sequence
  F2 primer for Foxn1
tccctaatccgatggctagctccag

SEQ ID NO: 42 - DNA, 23 bp, Artificial Sequence
  R1 primer for Foxn1
acgagcagctgaagttagcatgc

SEQ ID NO: 43 - DNA, 32 bp, Artificial Sequence
  R2 primer for Foxn1
ctactcaatgctcttagagctaccaggcttgc

SEQ ID NO: 44 - DNA, 20 bp, Artificial Sequence
  F primer for Prkdc
gactgttgtggggagggccg

SEQ ID NO: 45 - DNA, 24 bp, Artificial Sequence
  F2 primer for Prkdc
gggagggccgaaagtcttattttg

SEQ ID NO: 46 - DNA, 28 bp, Artificial Sequence
  R1 primer for Prkdc
cctgaagactgaagttggcagaagtgag

SEQ ID NO: 47 - DNA, 27 bp, Artificial Sequence
  R2 primer for Prkdc
ctttagggcttcttctctacaatcacg

SEQ ID NO: 48 - DNA, 38 bp, Artificial Sequence
  F primer for Foxn1
ctcggtgtgtagccctgacctcggtgtgtagccctgac

SEQ ID NO: 49 - DNA, 21 bp, Artificial Sequence
  R primer for Foxn1
agactggcctggaactcacag

SEQ ID NO: 50 - DNA, 23 bp, Artificial Sequence
  F primer for Foxn1
cactaaagcctgtcaggaagccg

SEQ ID NO: 51 - DNA, 21 bp, Artificial Sequence
  R primer for Foxn1
ctgtggagagcacacagcagc

SEQ ID NO: 52 - DNA, 19 bp, Artificial Sequence
  F primer for Foxn1
gctgcgacctgagaccatg

SEQ ID NO: 53 - DNA, 26 bp, Artificial Sequence
  R primer for Foxn1
cttcaatggcttcctgcttaggctac

SEQ ID NO: 54 - DNA, 23 bp, Artificial Sequence
  F primer for Foxn1
ggttcagatgaggccatcctttc

SEQ ID NO: 55 - DNA, 24 bp, Artificial Sequence
  R primer for Foxn1
cctgatctgcaggcttaacccttg

SEQ ID NO: 56 - DNA, 22 bp, Artificial Sequence
  F primer for Prkdc
ctcacctgcacatcacatgtgg

SEQ ID NO: 57 - DNA, 20 bp, Artificial Sequence
  R primer for Prkdc
ggcatccaccctatggggtc

SEQ ID NO: 58 - DNA, 25 bp, Artificial Sequence
  F primer for Prkdc
gccttgacctagagcttaaagagcc

SEQ ID NO: 59 - DNA, 25 bp, Artificial Sequence
  R primer for Prkdc
ggtcttgttagcaggaaggacactg

SEQ ID NO: 60 - DNA, 27 bp, Artificial Sequence
  F primer for Prkdc
aaaactctgcttgatgggatatgtggg

SEQ ID NO: 61 - DNA, 26 bp, Artificial Sequence
  R primer for Prkdc
ctctcactggttatctgtgctccttc

SEQ ID NO: 62 - DNA, 23 bp, Artificial Sequence
  F primer for Prkdc
ggatcaataggtggtgggggatg

SEQ ID NO: 63 - DNA, 27 bp, Artificial Sequence
  R primer for Prkdc
gtgaatgacacaatgtgacagcttcag

SEQ ID NO: 64 - DNA, 28 bp, Artificial Sequence
  F primer for Prkdc
cacaagacagacctctcaacattcagtc

SEQ ID NO: 65 - DNA, 32 bp, Artificial Sequence
  R primer for Prkdc
gtgcatgcatataatccattctgattgctctc

SEQ ID NO: 66 - DNA, 17 bp, Artificial Sequence
  F1 primer for Prkdc
gggaggcagaggcaggt

SEQ ID NO: 67 - DNA, 23 bp, Artificial Sequence
  F2 primer for Prkdc
ggatctctgtgagtttgaggcca

SEQ ID NO: 68 - DNA, 24 bp, Artificial Sequence
  R1 primer for Prkdc
gctccagaactcactcttaggctc

SEQ ID NO: 69 - DNA, 20 bp, Artificial Sequence
  Primer for Foxn1
ctactccctccgcagtctga

SEQ ID NO: 70 - DNA, 20 bp, Artificial Sequence
  Primer for Foxn1
ccaggcctaggttccaggta

SEQ ID NO: 71 - DNA, 20 bp, Artificial Sequence
  Primer for Prkdc
ccccagcattgcagatttcc

SEQ ID NO: 72 - DNA, 23 bp, Artificial Sequence
  Primer for Prkdc
agggcttcttctctacaatcacg

SEQ ID NO: 73 - DNA, 86 bp, Artificial Sequence
  BRI1 target 1
gaaattaatacgactcactataggtttgaaagatggaagcgcgggttttagagctagaaatagcaagttaaaataaggctagtccg

SEQ ID NO: 74 - DNA, 86 bp, Artificial Sequence
  BRI1 target 2
gaaattaatacgactcactataggtgaaactaaactggtccacagttttagagctagaaatagcaagttaaaataaggctagtccg

SEQ ID NO: 75 - DNA, 64 bp, Artificial Sequence
  Universal
aaaaaagcaccgactcggtgccactttttcaagttgataacggactagccttattttaacttgc

SEQ ID NO: 76 - DNA, 65 bp, Artificial Sequence
  Templates for crRNA
gaaattaatacgactcactataggnnnnnnnnnnnnnnnnnnnngttttagagctatgctgtttt

SEQ ID NO: 77 - DNA, 67 bp, Artificial Sequence
  tracrRNA
gaaattaatacgactcactataggaaccattcaaaacagcatagcaagttaaaataaggctagtccg

SEQ ID NO: 78 - DNA, 69 bp, Artificial Sequence
  tracrRNA
aaaaaaagcaccgactcggtgccactttttcaagttgataacggactagccttattttaacttgctatg

SEQ ID NO: 79 - DNA, 20 bp, Artificial Sequence
  Primer
ctccatggtgctatagagca

SEQ ID NO: 80 - DNA, 21 bp, Artificial Sequence
  Primer
gagccaagctctccatctagt

SEQ ID NO: 81 - DNA, 20 bp, Artificial Sequence
  Primer
gccctgtcaagagttgacac

SEQ ID NO: 82 - DNA, 22 bp, Artificial Sequence
  Primer
gcacagggtggaacaagatgga

SEQ ID NO: 83 - DNA, 24 bp, Artificial Sequence
  Primer
gccaggtacctatcgattgtcagg

SEQ ID NO: 84 - DNA, 21 bp, Artificial Sequence
  Primer
gagccaagctctccatctagt

SEQ ID NO: 85 - DNA, 20 bp, Artificial Sequence
  Primer
actctgactgggtcaccagc

SEQ ID NO: 86 - DNA, 20 bp, Artificial Sequence
  Primer
tatttggctggttgaaaggg

SEQ ID NO: 87 - DNA, 24 bp, Artificial Sequence
  Primer
aaagtcatgaaataaacacaccca

SEQ ID NO: 88 - DNA, 24 bp, Artificial Sequence
  Primer
ctgcattgatatggtagtaccatg

SEQ ID NO: 89 - DNA, 21 bp, Artificial Sequence
  Primer
gctgttcattgcaatggaatg

SEQ ID NO: 90 - DNA, 22 bp, Artificial Sequence
  Primer
atggagttggacatggccatgg

SEQ ID NO: 91 - DNA, 28 bp, Artificial Sequence
  Primer
actcactatccacagttcagcatttacc

SEQ ID NO: 92 - DNA, 23 bp, Artificial Sequence
  Primer
tggagatagctgtcagcaacttt

SEQ ID NO: 93 - DNA, 29 bp, Artificial Sequence
  Primer
caacaaagcaaaggtaaagttggtaatag

SEQ ID NO: 94 - DNA, 25 bp, Artificial Sequence
  Primer
ggtttcaggagatgtgttacaaggc

SEQ ID NO: 95 - DNA, 27 bp, Artificial Sequence
  Primer
gattgtgcaattcctatgcaatcggtc

SEQ ID NO: 96 - DNA, 25 bp, Artificial Sequence
  Primer
cactgggtacttaatctgtagcctc

SEQ ID NO: 97 - DNA, 23 bp, Artificial Sequence
  Primer
ggttccaagtcattcccagtagc

SEQ ID NO: 98 - DNA, 30 bp, Artificial Sequence
  Primer
catcactgcagttgtaggttataactatcc

SEQ ID NO: 99 - DNA, 26 bp, Artificial Sequence
  Primer
ttgaaaaccacagatctggttgaacc

SEQ ID NO: 100 - DNA, 22 bp, Artificial Sequence
  Primer
ggagtgccaagagaatatctgg

SEQ ID NO: 101 - DNA, 32 bp, Artificial Sequence
  Primer
ctgaaactggtttcaaaatattcgttttaagg

SEQ ID NO: 102 - DNA, 22 bp, Artificial Sequence
  Primer
gctctgtatgccctgtagtagg

SEQ ID NO: 103 - DNA, 22 bp, Artificial Sequence
  Primer
tttgcatctgaccttacctttg

SEQ ID NO: 104 - DNA, 23 bp, Artificial Sequence
  Target sequence of RGEN
aatgaccactacatcctcaaggg

SEQ ID NO: 105 - DNA, 23 bp, Artificial Sequence
  Target sequence of RGEN
agatgatgtctcatcatcagagg

SEQ ID NO: 106 - DNA, 4170 bp, Artificial Sequence
  Cas9-coding sequence in p3s-Cas9HC (humanized, C-term tagging, human cell experiments)
atggacaagaagtacagcatcggcctggacatcggtaccaacagcgtgggctgggccgtgatcaccgacgagtacaaggtgcccagcaagaagttcaaggtgctgggcaacaccgaccgccacagcatcaagaagaacctgatcggcgccctgctgttcgacagcggcgagaccgccgaggccacccgcctgaagcgcaccgcccgccgccgctacacccgccgcaagaaccgcatctgctacctgcaggagatcttcagcaacgagatggccaaggtggacgacagcttcttccaccgcctggaggagagcttcctggtggaggaggacaagaagcacgagcgccaccccatcttcggcaacatcgtggacgaggtggcctaccacgagaagtaccccaccatctaccacctgcgcaagaagctggtggacagcaccgacaaggccgacctgcgcctgatctacctggccctggcccacatgatcaagttccgcggccacttcctgatcgagggcgacctgaaccccgacaacagcgacgtggacaagctgttcatccagctggtgcagacctacaaccagctgttcgaggagaaccccatcaacgccagcggcgtggacgccaaggccatcctgagcgcccgcctgagcaagagccgccgcctggagaacctgatcgcccagctgcccggcgagaagaagaacggcctgttcggcaacctgatcgccctgagcctgggcctgacccccaacttcaagagcaacttcgacctggccgaggacgccaagctgcagctgagcaaggacacctacgacgacgacctggacaacctgctggcccagatcggcgaccagtacgccgacctgttcctggccgccaagaacctgagcgacgccatcctgctgagcgacatcctgcgcgtgaacaccgagatcaccaaggcccccctgagcgccagcatgatcaagcgctacgacgagcaccaccaggacctgaccctgctgaaggccctggtgcgccagcagctgcccgagaagtacaaggagatcttcttcgaccagagcaagaacggctacgccggctacatcgacggcggcgccagccaggaggagttctacaagttcatcaagcccatcctggagaagatggacggcaccgaggagctgctggtgaagctgaaccgcgaggacctgctgcgcaagcagcgcaccttcgacaacggcagcatcccccaccagatccacctgggcgagctgcacgccatcctgcgccgccaggaggacttctaccccttcctgaaggacaaccgcgagaagatcgagaagatcctgaccttccgcatcccctactacgtgggccccctggcccgcggcaacagccgcttcgcctggatgacccgcaagagcgaggagaccatcaccccctggaacttcgaggaggtggtggacaagggcgccagcgcccagagcttcatcgagcgcatgaccaacttcgacaagaacctgcccaacgagaaggtgctgcccaagcacagcctgctgtacgagtacttcaccgtgtacaacgagctgaccaaggtgaagtacgtgaccgagggcatgcgcaagcccgccttcctgagcggcgagcagaagaaggccatcgtggacctgctgttcaagaccaaccgcaaggtgaccgtgaagcagctgaaggaggactacttcaagaagatcgagtgcttcgacagcgtggagatcagcggcgtggaggaccgcttcaacgccagcctgggcacctaccacgacctgctgaagatcatcaaggacaaggacttcctggacaacgaggagaacgaggacatcctggaggacatcgtgctgaccctgaccctgttcgaggaccgcgagatgatcgaggagcgcctgaagacctacgcccacctgttcgacgacaaggtgatgaagcagctgaagcgccgccgctacaccggctggggccgcctgagccgcaagcttatcaacggcatccgcgacaagcagagcggcaagaccatcctggacttcctgaagagcgacggcttcgccaaccgcaacttcatgcagctgatccacgacgacagcctgaccttcaaggaggacatccagaaggcccaggtgagcggccagggcgacagcctgcacgagcacatcgccaacctggccggcagccccgccatcaagaagggcatcctgcagaccgtgaaggtggtggacgagctggtgaaggtgatgggccgccacaagcccgagaacatcgtgatcgagatggcccgcgagaaccagaccacccagaagggccagaagaacagccgcgagcgcatgaagcgcatcgaggagggcatcaaggagctgggcagccagatcctgaaggagcaccccgtggagaacacccagctgcagaacgagaagctgtacctgtactacctgcagaacggccgcgacatgtacgtggaccaggagctggacatcaaccgcctgagcgactacgacgtggaccacatcgtgccccagagcttcctgaaggacgacagcatcgacaacaaggtgctgacccgcagcgacaagaaccgcggcaagagcgacaacgtgcccagcgaggaggtggtgaagaagatgaagaactactggcgccagctgctgaacgccaagctgatcacccagcgcaagttcgacaacctgaccaaggccgagcgcggcggcctgagcgagctggacaaggccggcttcatcaagcgccagctggtggagacccgccagatcaccaagcacgtggcccagatcctggacagccgcatgaacaccaagtacgacgagaacgacaagctgatccgcgaggtgaaggtgatcaccctgaagagcaagctggtgagcgacttccgcaaggacttccagttctacaaggtgcgcgagatcaacaactaccaccacgcccacgacgcctacctgaacgccgtggtgggcaccgccctgatcaagaagtaccccaagctggagagcgagttcgtgtacggcgactacaaggtgtacgacgtgcgcaagatgatcgccaagagcgagcaggagatcggcaaggccaccgccaagtacttcttctacagcaacatcatgaacttcttcaagaccgagatcaccctggccaacggcgagatccgcaagcgccccctgatcgagaccaacggcgagaccggcgagatcgtgtgggacaagggccgcgacttcgccaccgtgcgcaaggtgctgagcatgccccaggtgaacatcgtgaagaagaccgaggtgcagaccggcggcttcagcaaggagagcatcctgcccaagcgcaacagcgacaagctgatcgcccgcaagaaggactgggaccccaagaagtacggcggcttcgacagccccaccgtggcctacagcgtgctggtggtggccaaggtggagaagggcaagagcaagaagctgaagagcgtgaaggagctgctgggcatcaccatcatggagcgcagcagcttcgagaagaaccccatcgacttcctggaggccaagggctacaaggaggtgaagaaggacctgatcatcaagctgcccaagtacagcctgttcgagctggagaacggccgcaagcgcatgctggccagcgccggcgagctgcagaagggcaacgagctggccctgcccagcaagtacgtgaacttcctgtacctggccagccactacgagaagctgaagggcagccccgaggacaacgagcagaagcagctgttcgtggagcagcacaagcactacctggacgagatcatcgagcagatcagcgagttcagcaagcgcgtgatcctggccgacgccaacctggacaaggtgctgagcgcctacaacaagcaccgcgacaagcccatccgcgagcaggccgagaacatcatccacctgttcaccctgaccaacctgggcgcccccgccgccttcaagtacttcgacaccaccatcgaccgcaagcgctacaccagcaccaaggaggtgctggacgccaccctgatccaccagagcatcaccggtctgtacgagacccgcatcgacctgagccagctgggcggcgacggcggctccggacctccaaagaaaaagagaaaagtatacccctacgacgtgcccgactacgcctaa

SEQ ID NO: 107 - DNA, 4194 bp, Artificial Sequence
  Cas9 coding sequence in p3s-Cas9HN (humanized codon, N-term tagging (underlined), human cell experiments)
atggtgtacccctacgacgtgcccgactacgccgaattgcctccaaaaaagaagagaaaggtagggatccgaattcccggggaaaaaccggacaagaagtacagcatcggcctggacatcggtaccaacagcgtgggctgggccgtgatcaccgacgagtacaaggtgcccagcaagaagttcaaggtgctgggcaacaccgaccgccacagcatcaagaagaacctgatcggcgccctgctgttcgacagcggcgagaccgccgaggccacccgcctgaagcgcaccgcccgccgccgctacacccgccgcaagaaccgcatctgctacctgcaggagatcttcagcaacgagatggccaaggtggacgacagcttcttccaccgcctggaggagagcttcctggtggaggaggacaagaagcacgagcgccaccccatcttcggcaacatcgtggacgaggtggcctaccacgagaagtaccccaccatctaccacctgcgcaagaagctggtggacagcaccgacaaggccgacctgcgcctgatctacctggccctggcccacatgatcaagttccgcggccacttcctgatcgagggcgacctgaaccccgacaacagcgacgtggacaagctgttcatccagctggtgcagacctacaaccagctgttcgaggagaaccccatcaacgccagcggcgtggacgccaaggccatcctgagcgcccgcctgagcaagagccgccgcctggagaacctgatcgcccagctgcccggcgagaagaagaacggcctgttcggcaacctgatcgccctgagcctgggcctgacccccaacttcaagagcaacttcgacctggccgaggacgccaagctgcagctgagcaaggacacctacgacgacgacctggacaacctgctggcccagatcggcgaccagtacgccgacctgttcctggccgccaagaacctgagcgacgccatcctgctgagcgacatcctgcgcgtgaacaccgagatcaccaaggcccccctgagcgccagcatgatcaagcgctacgacgagcaccaccaggacctgaccctgctgaaggccctggtgcgccagcagctgcccgagaagtacaaggagatcttcttcgaccagagcaagaacggctacgccggctacatcgacggcggcgccagccaggaggagttctacaagttcatcaagcccatcctggagaagatggacggcaccgaggagctgctggtgaagctgaaccgcgaggacctgctgcgcaagcagcgcaccttcgacaacggcagcatcccccaccagatccacctgggcgagctgcacgccatcctgcgccgccaggaggacttctaccccttcctgaaggacaaccgcgagaagatcgagaagatcctgaccttccgcatcccctactacgtgggccccctggcccgcggcaacagccgcttcgcctggatgacccgcaagagcgaggagaccatcaccccctggaacttcgaggaggtggtggacaagggcgccagcgcccagagcttcatcgagcgcatgaccaacttcgacaagaacctgcccaacgagaaggtgctgcccaagcacagcctgctgtacgagtacttcaccgtgtacaacgagctgaccaaggtgaagtacgtgaccgagggcatgcgcaagcccgccttcctgagcggcgagcagaagaaggccatcgtggacctgctgttcaagaccaaccgcaaggtgaccgtgaagcagctgaaggaggactacttcaagaagatcgagtgcttcgacagcgtggagatcagcggcgtggaggaccgcttcaacgccagcctgggcacctaccacgacctgctgaagatcatcaaggacaaggacttcctggacaacgaggagaacgaggacatcctggaggacatcgtgctgaccctgaccctgttcgaggaccgcgagatgatcgaggagcgcctgaagacctacgcccacctgttcgacgacaaggtgatgaagcagctgaagcgccgccgctacaccggctggggccgcctgagccgcaagcttatcaacggcatccgcgacaagcagagcggcaagaccatcctggacttcctgaagagcgacggcttcgccaaccgcaacttcatgcagctgatccacgacgacagcctgaccttcaaggaggacatccagaaggcccaggtgagcggccagggcgacagcctgcacgagcacatcgccaacctggccggcagccccgccatcaagaagggcatcctgcagaccgtgaaggtggtggacgagctggtgaaggtgatgggccgccacaagcccgagaacatcgtgatcgagatggcccgcgagaaccagaccacccagaagggccagaagaacagccgcgagcgcatgaagcgcatcgaggagggcatcaaggagctgggcagccagatcctgaaggagcaccccgtggagaacacccagctgcagaacgagaagctgtacctgtactacctgcagaacggccgcgacatgtacgtggaccaggagctggacatcaaccgcctgagcgactacgacgtggaccacatcgtgccccagagcttcctgaaggacgacagcatcgacaacaaggtgctgacccgcagcgacaagaaccgcggcaagagcgacaacgtgcccagcgaggaggtggtgaagaagatgaagaactactggcgccagctgctgaacgccaagctgatcacccagcgcaagttcgacaacctgaccaaggccgagcgcggcggcctgagcgagctggacaaggccggcttcatcaagcgccagctggtggagacccgccagatcaccaagcacgtggcccagatcctggacagccgcatgaacaccaagtacgacgagaacgacaagctgatccgcgaggtgaaggtgatcaccctgaagagcaagctggtgagcgacttccgcaaggacttccagttctacaaggtgcgcgagatcaacaactaccaccacgcccacgacgcctacctgaacgccgtggtgggcaccgccctgatcaagaagtaccccaagctggagagcgagttcgtgtacggcgactacaaggtgtacgacgtgcgcaagatgatcgccaagagcgagcaggagatcggcaaggccaccgccaagtacttcttctacagcaacatcatgaacttcttcaagaccgagatcaccctggccaacggcgagatccgcaagcgccccctgatcgagaccaacggcgagaccggcgagatcgtgtgggacaagggccgcgacttcgccaccgtgcgcaaggtgctgagcatgccccaggtgaacatcgtgaagaagaccgaggtgcagaccggcggcttcagcaaggagagcatcctgcccaagcgcaacagcgacaagctgatcgcccgcaagaaggactgggaccccaagaagtacggcggcttcgacagccccaccgtggcctacagcgtgctggtggtggccaaggtggagaagggcaagagcaagaagctgaagagcgtgaaggagctgctgggcatcaccatcatggagcgcagcagcttcgagaagaaccccatcgacttcctggaggccaagggctacaaggaggtgaagaaggacctgatcatcaagctgcccaagtacagcctgttcgagctggagaacggccgcaagcgcatgctggccagcgccggcgagctgcagaagggcaacgagctggccctgcccagcaagtacgtgaacttcctgtacctggccagccactacgagaagctgaagggcagccccgaggacaacgagcagaagcagctgttcgtggagcagcacaagcactacctggacgagatcatcgagcagatcagcgagttcagcaagcgcgtgatcctggccgacgccaacctggacaaggtgctgagcgcctacaacaagcaccgcgacaagcccatccgcgagcaggccgagaacatcatccacctgttcaccctgaccaacctgggcgcccccgccgccttcaagtacttcgacaccaccatcgaccgcaagcgctacaccagcaccaaggaggtgctggacgccaccctgatccaccagagcatcaccggtctgtacgagacccgcatcgacctgagccagctgggcggcgactaa

SEQ ID NO: 108 - DNA, 4107 bp, Artificial Sequence
  Cas9-coding sequence in Streptococcus pyogenes
atggataagaaatactcaataggcttagatatcggcacaaatagcgtcggatgggcggtgatcactgatgaatataaggttccgtctaaaaagttcaaggttctgggaaatacagaccgccacagtatcaaaaaaaatcttataggggctcttttatttgacagtggagagacagcggaagcgactcgtctcaaacggacagctcgtagaaggtatacacgtcggaagaatcgtatttgttatctacaggagattttttcaaatgagatggcgaaagtagatgatagtttctttcatcgacttgaagagtcttttttggtggaagaagacaagaagcatgaacgtcatcctatttttggaaatatagtagatgaagttgcttatcatgagaaatatccaactatctatcatctgcgaaaaaaattggtagattctactgataaagcggatttgcgcttaatctatttggccttagcgcatatgattaagtttcgtggtcattttttgattgagggagatttaaatcctgataatagtgatgtggacaaactatttatccagttggtacaaacctacaatcaattatttgaagaaaaccctattaacgcaagtggagtagatgctaaagcgattctttctgcacgattgagtaaatcaagacgattagaaaatctcattgctcagctccccggtgagaagaaaaatggcttatttgggaatctcattgctttgtcattgggtttgacccctaattttaaatcaaattttgatttggcagaagatgctaaattacagctttcaaaagatacttacgatgatgatttagataatttattggcgcaaattggagatcaatatgctgatttgtttttggcagctaagaatttatcagatgctattttactttcagatatcctaagagtaaatactgaaataactaaggctcccctatcagcttcaatgattaaacgctacgatgaacatcatcaagacttgactcttttaaaagctttagttcgacaacaacttccagaaaagtataaagaaatcttttttgatcaatcaaaaaacggatatgcaggttatattgatgggggagctagccaagaagaattttataaatttatcaaaccaattttagaaaaaatggatggtactgaggaattattggtgaaactaaatcgtgaagatttgctgcgcaagcaacggacctttgacaacggctctattccccatcaaattcacttgggtgagctgcatgctattttgagaagacaagaagacttttatccatttttaaaagacaatcgtgagaagattgaaaaaatcttgacttttcgaattccttattatgttggtccattggcgcgtggcaatagtcgttttgcatggatgactcggaagtctgaagaaacaattaccccatggaattttgaagaagttgtcgataaaggtgcttcagctcaatcatttattgaacgcatgacaaactttgataaaaatcttccaaatgaaaaagtactaccaaaacatagtttgctttatgagtattttacggtttataacgaattgacaaaggtcaaatatgttactgaaggaatgcgaaaaccagcatttctttcaggtgaacagaagaaagccattgttgatttactcttcaaaacaaatcgaaaagtaaccgttaagcaattaaaagaagattatttcaaaaaaatagaatgttttgatagtgttgaaatttcaggagttgaagatagatttaatgcttcattaggtacctaccatgatttgctaaaaattattaaagataaagattttttggataatgaagaaaatgaagatatcttagaggatattgttttaacattgaccttatttgaagatagggagatgattgaggaaagacttaaaacatatgctcacctctttgatgataaggtgatgaaacagcttaaacgtcgccgttatactggttggggacgtttgtctcgaaaattgattaatggtattagggataagcaatctggcaaaacaatattagattttttgaaatcagatggttttgccaatcgcaattttatgcagctgatccatgatgatagtttgacatttaaagaagacattcaaaaagcacaagtgtctggacaaggcgatagtttacatgaacatattgcaaatttagctggtagccctgctattaaaaaaggtattttacagactgtaaaagttgttgatgaattggtcaaagtaatggggcggcataagccagaaaatatcgttattgaaatggcacgtgaaaatcagacaactcaaaagggccagaaaaattcgcgagagcgtatgaaacgaatcgaagaaggtatcaaagaattaggaagtcagattcttaaagagcatcctgttgaaaatactcaattgcaaaatgaaaagctctatctctattatctccaaaatggaagagacatgtatgtggaccaagaattagatattaatcgtttaagtgattatgatgtcgatcacattgttccacaaagtttccttaaagacgattcaatagacaataaggtcttaacgcgttctgataaaaatcgtggtaaatcggataacgttccaagtgaagaagtagtcaaaaagatgaaaaactattggagacaacttctaaacgccaagttaatcactcaacgtaagtttgataatttaacgaaagctgaacgtggaggtttgagtgaacttgataaagctggttttatcaaacgccaattggttgaaactcgccaaatcactaagcatgtggcacaaattttggatagtcgcatgaatactaaatacgatgaaaatgataaacttattcgagaggttaaagtgattaccttaaaatctaaattagtttctgacttccgaaaagatttccaattctataaagtacgtgagattaacaattaccatcatgcccatgatgcgtatctaaatgccgtcgttggaactgctttgattaagaaatatccaaaacttgaatcggagtttgtctatggtgattataaagtttatgatgttcgtaaaatgattgctaagtctgagcaagaaataggcaaagcaaccgcaaaatatttcttttactctaatatcatgaacttcttcaaaacagaaattacacttgcaaatggagagattcgcaaacgccctctaatcgaaactaatggggaaactggagaaattgtctgggataaagggcgagattttgccacagtgcgcaaagtattgtccatgccccaagtcaatattgtcaagaaaacagaagtacagacaggcggattctccaaggagtcaattttaccaaaaagaaattcggacaagcttattgctcgtaaaaaagactgggatccaaaaaaatatggtggttttgatagtccaacggtagcttattcagtcctagtggttgctaaggtggaaaaagggaaatcgaagaagttaaaatccgttaaagagttactagggatcacaattatggaaagaagttcctttgaaaaaaatccgattgactttttagaagctaaaggatataaggaagttaaaaaagacttaatcattaaactacctaaatatagtctttttgagttagaaaacggtcgtaaacggatgctggctagtgccggagaattacaaaaaggaaatgagctggctctgccaagcaaatatgtgaattttttatatttagctagtcattatgaaaagttgaagggtagtccagaagataacgaacaaaaacaattgtttgtggagcagcataagcattatttagatgagattattgagcaaatcagtgaattttctaagcgtgttattttagcagatgccaatttagataaagttcttagtgcatataacaaacatagagacaaaccaatacgtgaacaagcagaaaatattattcatttatttacgttgacgaatcttggagctcccgctgcttttaaatattttgatacaacaattgatcgtaaacgatatacgtctacaaaagaagttttagatgccactcttatccatcaatccatcactggtctttatgaaacacgcattgatttgagtcagctaggaggtgactaa

SEQ ID NO: 109 - protein, 1368 aa, Artificial Sequence [sequence omitted]

SEQ ID NO: 110 - DNA, 4221 bp, Artificial Sequence
  Cas9-coding sequence in pET-Cas9N3T for the production of recombinant Cas9 protein in E. coli (humanized codon; hexa-His-tag and a nuclear localization signal at the N terminus)
atgggcagcagccatcatcatcatcatcatgtgtacccctacgacgtgcccgactacgccgaattgcctccaaaaaagaagagaaaggtagggatcgagaacctgtacttccagggcgacaagaagtacagcatcggcctggacatcggtaccaacagcgtgggctgggccgtgatcaccgacgagtacaaggtgcccagcaagaagttcaaggtgctgggcaacaccgaccgccacagcatcaagaagaacctgatcggcgccctgctgttcgacagcggcgagaccgccgaggccacccgcctgaagcgcaccgcccgccgccgctacacccgccgcaagaaccgcatctgctacctgcaggagatcttcagcaacgagatggccaaggtggacgacagcttcttccaccgcctggaggagagcttcctggtggaggaggacaagaagcacgagcgccaccccatcttcggcaacatcgtggacgaggtggcctaccacgagaagtaccccaccatctaccacctgcgcaagaagctggtggacagcaccgacaaggccgacctgcgcctgatctacctggccctggcccacatgatcaagttccgcggccacttcctgatcgagggcgacctgaaccccgacaacagcgacgtggacaagctgttcatccagctggtgcagacctacaaccagctgttcgaggagaaccccatcaacgccagcggcgtggacgccaaggccatcctgagcgcccgcctgagcaagagccgccgcctggagaacctgatcgcccagctgcccggcgagaagaagaacggcctgttcggcaacctgatcgccctgagcctgggcctgacccccaacttcaagagcaacttcgacctggccgaggacgccaagctgcagctgagcaaggacacctacgacgacgacctggacaacctgctggcccagatcggcgaccagtacgccgacctgttcctggccgccaagaacctgagcgacgccatcctgctgagcgacatcctgcgcgtgaacaccgagatcaccaaggcccccctgagcgccagcatgatcaagcgctacgacgagcaccaccaggacctgaccctgctgaaggccctggtgcgccagcagctgcccgagaagtacaaggagatcttcttcgaccagagcaagaacggctacgccggctacatcgacggcggcgccagccaggaggagttctacaagttcatcaagcccatcctggagaagatggacggcaccgaggagctgctggtgaagctgaaccgcgaggacctgctgcgcaagcagcgcaccttcgacaacggcagcatcccccaccagatccacctgggcgagctgcacgccatcctgcgccgccaggaggacttctaccccttcctgaaggacaaccgcgagaagatcgagaagatcctgaccttccgcatcccctactacgtgggccccctggcccgcggcaacagccgcttcgcctggatgacccgcaagagcgaggagaccatcaccccctggaacttcgaggaggtggtggacaagggcgccagcgcccagagcttcatcgagcgcatgaccaacttcgacaagaacctgcccaacgagaaggtgctgcccaagcacagcctgctgtacgagtacttcaccgtgtacaacgagctgaccaaggtgaagtacgtgaccgagggcatgcgcaagcccgccttcctgagcggcgagcagaagaaggccatcgtggacctgctgttcaagaccaaccgcaaggtgaccgtgaagcagctgaaggaggactacttcaagaagatcgagtgcttcgacagcgtggagatcagcggcgtggaggaccgcttcaacgccagcctgggcacctaccacgacctgctgaagatcatcaaggacaaggacttcctggacaacgaggagaacgaggacatcctggaggacatcgtgctgaccctgaccctgttcgaggaccgcgagatgatcgaggagcgcctgaagacctacgcccacctgttcgacgacaaggtgatgaagcagctgaagcgccgccgctacaccggctggggccgcctgagccgcaagcttatcaacggcatccgcgacaagcagagcggcaagaccatcctggacttcctgaagagcgacggcttcgccaaccgcaacttcatgcagctgatccacgacgacagcctgaccttcaaggaggacatccagaaggcccaggtgagcggccagggcgacagcctgcacgagcacatcgccaacctggccggcagccccgccatcaagaagggcatcctgcagaccgtgaaggtggtggacgagctggtgaaggtgatgggccgccacaagcccgagaacatcgtgatcgagatggcccgcgagaaccagaccacccagaagggccagaagaacagccgcgagcgcatgaagcgcatcgaggagggcatcaaggagctgggcagccagatcctgaaggagcaccccgtggagaacacccagctgcagaacgagaagctgtacctgtactacctgcagaacggccgcgacatgtacgtggaccaggagctggacatcaaccgcctgagcgactacgacgtggaccacatcgtgccccagagcttcctgaaggacgacagcatcgacaacaaggtgctgacccgcagcgacaagaaccgcggcaagagcgacaacgtgcccagcgaggaggtggtgaagaagatgaagaactactggcgccagctgctgaacgccaagctgatcacccagcgcaagttcgacaacctgaccaaggccgagcgcggcggcctgagcgagctggacaaggccggcttcatcaagcgccagctggtggagacccgccagatcaccaagcacgtggcccagatcctggacagccgcatgaacaccaagtacgacgagaacgacaagctgatccgcgaggtgaaggtgatcaccctgaagagcaagctggtgagcgacttccgcaaggacttccagttctacaaggtgcgcgagatcaacaactaccaccacgcccacgacgcctacctgaacgccgtggtgggcaccgccctgatcaagaagtaccccaagctggagagcgagttcgtgtacggcgactacaaggtgtacgacgtgcgcaagatgatcgccaagagcgagcaggagatcggcaaggccaccgccaagtacttcttctacagcaacatcatgaacttcttcaagaccgagatcaccctggccaacggcgagatccgcaagcgccccctgatcgagaccaacggcgagaccggcgagatcgtgtgggacaagggccgcgacttcgccaccgtgcgcaaggtgctgagcatgccccaggtgaacatcgtgaagaagaccgaggtgcagaccggcggcttcagcaaggagagcatcctgcccaagcgcaacagcgacaagctgatcgcccgcaagaaggactgggaccccaagaagtacggcggcttcgacagccccaccgtggcctacagcgtgctggtggtggccaaggtggagaagggcaagagcaagaagctgaagagcgtgaaggagctgctgggcatcaccatcatggagcgcagcagcttcgagaagaaccccatcgacttcctggaggccaagggctacaaggaggtgaagaaggacctgatcatcaagctgcccaagtacagcctgttcgagctggagaacggccgcaagcgcatgctggccagcgccggcgagctgcagaagggcaacgagctggccctgcccagcaagtacgtgaacttcctgtacctggccagccactacgagaagctgaagggcagccccgaggacaacgagcagaagcagctgttcgtggagcagcacaagcactacctggacgagatcatcgagcagatcagcgagttcagcaagcgcgtgatcctggccgacgccaacctggacaaggtgctgagcgcctacaacaagcaccgcgacaagcccatccgcgagcaggccgagaacatcatccacctgttcaccctgaccaacctgggcgcccccgccgccttcaagtacttcgacaccaccatcgaccgcaagcgctacaccagcaccaaggaggtgctggacgccaccctgatccaccagagcatcaccggtctgtacgagacccgcatcgacctgagccagctgggcggcgactaa

SEQ ID NO: 111 - protein, 1406 aa, Artificial Sequence
  Amino acid sequence of Cas9 (pET-Cas9N3T)
MGSSHHHHHHVYPYDVPDYAELPPKKKRKVGIENLYFQGDKKYSIGLDIGTNSVGWAVITDEYKVPSKKFKVLGNTDRHSIKKNLIGALLFDSGETAEATRLKRTARRRYTRRKNRICYLQEIFSNEMAKVDDSFFHRLEESFLVEEDKKHERHPIFGNIVDEVAYHEKYPTIYHLRKKLVDSTDKADLRLIYLALAHMIKFRGHFLIEGDLNPDNSDVDKLFIQLVQTYNQLFEENPINASGVDAKAILSARLSKSRRLENLIAQLPGEKKNGLFGNLIALSLGLTPNFKSNFDLAEDAKLQLSKDTYDDDLDNLLAQIGDQYADLFLAAKNLSDAILLSDILRVNTEITKAPLSASMIKRYDEHHQDLTLLKALVRQQLPEKYKEIFFDQSKNGYAGYIDGGASQEEFYKFIKPILEKMDGTEELLVKLNREDLLRKQRTFDNGSIPHQIHLGELHAILRRQEDFYPFLKDNREKIEKILTFRIPYYVGPLARGNSRFAWMTRKSEETITPWNFEEVVDKGASAQSFIERMTNFDKNLPNEKVLPKHSLLYEYFTVYNELTKVKYVTEGMRKPAFLSGEQKKAIVDLLFKTNRKVTVKQLKEDYFKKIECFDSVEISGVEDRFNASLGTYHDLLKIIKDKDFLDNEENEDILEDIVLTLTLFEDREMIEERLKTYAHLFDDKVMKQLKRRRYTGWGRLSRKLINGIRDKQSGKTILDFLKSDGFANRNFMQLIHDDSLTFKEDIQKAQVSGQGDSLHEHIANLAGSPAIKKGILQTVKVVDELVKVMGRHKPENIVIEMARENQTTQKGQKNSRERMKRIEEGIKELGSQILKEHPVENTQLQNEKLYLYYLQNGRDMYVDQELDINRLSDYDVDHIVPQSFLKDDSIDNKVLTRSDKNRGKSDNVPSEEVVKKMKNYWRQLLNAKLITQRKFDNLTKAERGGLSELDKAGFIKRQLVETRQITKHVAQILDSRMNTKYDENDKLIREVKVITLKSKLVSDFRKDFQFYKVREINNYHHAHDAYLNAVVGTALIKKYPKLESEFVYGDYKVYDVRKMIAKSEQEIGKATAKYFFYSNIMNFFKTEITLANGEIRKRPLIETNGETGEIVWDKGRDFATVRKVLSMPQVNIVKKTEVQTGGFSKESILPKRNSDKLIARKKDWDPKKYGGFDSPTVAYSVLVVAKVEKGKSKKLKSVKELLGITIMERSSFEKNPIDFLEAKGYKEVKKDLIIKLPKYSLFELENGRKRMLASAGELQKGNELALPSKYVNFLYLASHYEKLKGSPEDNEQKQLFVEQHKHYLDEIIEQISEFSKRVILADANLDKVLSAYNKHRDKPIREQAENIIHLFTLTNLGAPAAFKYFDTTIDRKRYTSTKEVLDATLIHQSITGLYETRIDLSQLGGD